European Patent Application EP 4 289 947 A1, published December 13, 2023. Title: HIGH-STEREOSELECTIVITY R TRANSKETOLASE MUTANT, AND ENCODING GENE AND USE THEREOF. Applicant: ZHEJIANG APELOA KANGYU PHARMACEUTICAL CO., LTD. APELOA PHARMACEUTICAL CO., LTD. The sequence listing filed with the application follows.

SEQUENCE LISTING (19 sequences)

SEQ ID NO: 1 - protein, 663 aa, Artificial Sequence
  EcTK1_YYH amino acid sequence
MSSRKELANAIRALSMDAVQKAKSGYPGAPMGMADIAEVLWRDFLKHNPQNPSWADRDRFVLSNGHGSMLIYSLLHLTGYDLPMEELKNFRQLHSKTPGHPEVGYTAGVETTTGPLGQGIANAVGMAIAEKTLAAQFNRPGHDIVDHYTYAFMGDGCMMEGISHEVCSLAGTLKLGKLIAFYDDNGISIDGHVEGWFTDDTAMRFEAYGWHVIRDIDGHDAASIKRAVEEARAVTDKPSLLMCKTIIGFGSPNKAGTHDSHGAPLGDAEIALTREQLGWKYAPFEIPSEIYAQWDAKEAGQAKESAWNEKFAAYAKAYPQEAAEFTRRMKGEMPSDFDAKAKEFIAKLQANPAKIASRKASQNAIEAFGPLLPEFLGGSADLAPYNLTLWSGSKAINEDAAGNYIHYGVREFGMTAIANGISLHGGFLPYTSTYLMFVEYARNAVRMAALMKQRQVMVYTHDSIGHGETGPTHQPVEQVASLRVTPNMSTWRPCDQVESAVAWKYGVERQDGPTALILSQQNLAQQERTEEQLANIARGGYVLKDCAGQPELIFIATGSEVELAVAAYEKLTAEGVKARVVSMPSTDAFDKQDAAYRESVLPKAVTARVAVEAGIADYWYKYVGLNGAIVGMTTFGESAPAELLFEEFGFTVDNVVAKAKELL

SEQ ID NO: 2 - DNA, 1992 bp, Artificial Sequence
  EcTK1_YYH nucleotide sequence
atgtcctcacgtaaagagcttgccaatgctattcgtgcgctgagcatggacgcagtacagaaagccaaatccggttatccgggtgcccctatgggtatggctgacattgccgaagtcctgtggcgtgatttcctgaaacacaacccgcagaatccgtcctgggctgaccgtgaccgcttcgtgctgtccaacggccacggctccatgctgatctacagcctgctgcacctcaccggttacgatctgccgatggaagaactgaaaaacttccgtcagctgcactctaaaactccgggtcacccggaagtgggttacaccgctggtgtggaaaccaccaccggtccgctgggtcagggtattgccaacgcagtcggtatggcgattgcagaaaaaacgctggcggcgcagtttaaccgtccgggccacgacattgtcgaccactacacctacgccttcatgggcgacggctgcatgatggaaggcatctcccacgaagtttgctctctggcgggtacgctgaagttgggtaaactgattgcattctacgatgacaacggtatttctatcgatggtcacgttgaaggctggttcaccgacgacaccgcaatgcgtttcgaagcttacggctggcacgttattcgcgacatcgacggtcatgacgcggcatctatcaaacgcgcagtagaagaagcgcgcgcagtgactgacaaaccttccctgctgatgtgcaaaaccatcatcggtttcggttccccgaacaaagccggtacccacgactcccacggtgcgccgctgggcgacgctgaaattgccctgacccgcgaacaactgggctggaaatatgcgccgttcgaaatcccgtctgaaatctatgctcagtgggatgcgaaagaagcaggccaggcgaaagaatccgcatggaacgagaaattcgctgcttacgcgaaagcttatccgcaggaagccgctgaatttacccgccgtatgaaaggcgaaatgccgtctgacttcgacgctaaagcgaaagagttcatcgctaaactgcaggctaatccggcgaaaatcgccagccgtaaagcgtctcagaatgctatcgaagcgttcggtccgctgttgccggaattcctcggcggttctgctgacctggcgccgtataacctgaccctgtggtctggttctaaagcaatcaacgaagatgctgcgggtaactacatccactacggtgttcgcgagttcggtatgaccgcgattgctaacggtatctccctgcacggtggcttcctgccgtacacctccacctatctgatgttcgtggaatacgcacgtaacgccgtacgtatggctgcgctgatgaaacagcgtcaggtgatggtttacacccacgactccatcggtcatggcgaaaccggcccgactcaccagccggttgagcaggtcgcttctctgcgcgtaaccccgaacatgtctacatggcgtccgtgtgaccaggttgaatccgcggtcgcgtggaaatacggtgttgagcgtcaggacggcccgaccgcactgatcctctcccaacagaacctggcgcagcaggaacgaactgaagagcaactggcaaacatcgcgcgcggtggttatgtgctgaaagactgcgccggtcagccggaactgattttcatcgctaccggttcagaagttgaactggctgttgctgcctacgaaaaactgactgccgaaggcgtgaaagcgcgcgtggtgtccatgccgtctaccgacgcatttgacaagcaggatgctgcttaccgtgaatccgtactgccgaaagcggttactgcacgcgttgctgtagaagcgggtattgctgactactggtacaagtatgttggcctgaacggtgctatcgtcggtatgaccaccttcggtgaatctgctccggcagagctgctgtttgaagagttcggcttcactgttgataacgttgttgcgaaagcaaaagaactgctgtaa

SEQ ID NO: 3 - DNA, 7288 bp, Artificial Sequence
  pET28a-TK template nucleotide sequence
tggcgaatgggacgcgccctgtagcggcgcattaagcgcggcgggtgtggtggttacgcgcagcgtgaccgctacacttgccagcgccctagcgcccgctcctttcgctttcttcccttcctttctcgccacgttcgccggctttccccgtcaagctctaaatcgggggctccctttagggttccgatttagtgctttacggcacctcgaccccaaaaaacttgattagggtgatggttcacgtagtgggccatcgccctgatagacggtttttcgccctttgacgttggagtccacgttctttaatagtggactcttgttccaaactggaacaacactcaaccctatctcggtctattcttttgatttataagggattttgccgatttcggcctattggttaaaaaatgagctgatttaacaaaaatttaacgcgaattttaacaaaatattaacgtttacaatttcaggtggcacttttcggggaaatgtgcgcggaacccctatttgtttatttttctaaatacattcaaatatgtatccgctcatgaattaattcttagaaaaactcatcgagcatcaaatgaaactgcaatttattcatatcaggattatcaataccatatttttgaaaaagccgtttctgtaatgaaggagaaaactcaccgaggcagttccataggatggcaagatcctggtatcggtctgcgattccgactcgtccaacatcaatacaacctattaatttcccctcgtcaaaaataaggttatcaagtgagaaatcaccatgagtgacgactgaatccggtgagaatggcaaaagtttatgcatttctttccagacttgttcaacaggccagccattacgctcgtcatcaaaatcactcgcatcaaccaaaccgttattcattcgtgattgcgcctgagcgagacgaaatacgcgatcgctgttaaaaggacaattacaaacaggaatcgaatgcaaccggcgcaggaacactgccagcgcatcaacaatattttcacctgaatcaggatattcttctaatacctggaatgctgttttcccggggatcgcagtggtgagtaaccatgcatcatcaggagtacggataaaatgcttgatggtcggaagaggcataaattccgtcagccagtttagtctgaccatctcatctgtaacatcattggcaacgctacctttgccatgtttcagaaacaactctggcgcatcgggcttcccatacaatcgatagattgtcgcacctgattgcccgacattatcgcgagcccatttatacccatataaatcagcatccatgttggaatttaatcgcggcctagagcaagacgtttcccgttgaatatggctcataacaccccttgtattactgtttatgtaagcagacagttttattgttcatgaccaaaatcccttaacgtgagttttcgttccactgagcgtcagaccccgtagaaaagatcaaaggatcttcttgagatcctttttttctgcgcgtaatctgctgcttgcaaacaaaaaaaccaccgctaccagcggtggtttgtttgccggatcaagagctaccaactctttttccgaaggtaactggcttcagcagagcgcagataccaaatactgtccttctagtgtagccgtagttaggccaccacttcaagaactctgtagcaccgcctacatacctcgctctgctaatcctgttaccagtggctgctgccagtggcgataagtcgtgtcttaccgggttggactcaagacgatagttaccggataaggcgcagcggtcgggctgaacggggggttcgtgcacacagcccagcttggagcgaacgacctacaccgaactgagatacctacagcgtgagctatgagaaagcgccacgcttcccgaagggagaaaggcggacaggtatccggtaagcggcagggtcggaacaggagagcgcacgagggagcttccagggggaaacgcctggtatctttatagtcctgtcgggtttcgccacctctgacttgagcgtcgatttttgtgatgctcgtcaggggggcggagcctatggaaaaacgccagcaacgcggcctttttacggttcctggccttttgctggccttttgctcacatgttctttcctgcgttatcccctgattctgtggataaccgtattaccgcctttgagtgagctgataccgctcgccgcagccgaacgaccgagcgcagcgagtcagtgagcgaggaagcggaagagcgcctgatgcggtattttctccttacgcatctgtgcggtatttcacaccgcatatatggtgcactctcagtacaatctgctctgatgccgcatagttaagccagtatacactccgctatcgctacgtgactgggtcatggctgcgccccgacacccgccaacacccgctgacgcgccctgacgggcttgtctgctcccggcatccgcttacagacaagctgtgaccgtctccgggagctgcatgtgtcagaggttttcaccgtcatcaccgaaacgcgcgaggcagctgcggtaaagctcatcagcgtggtcgtgaagcgattcacagatgtctgcctgttcatccgcgtccagctcgttgagtttctccagaagcgttaatgtctggcttctgataaagcgggccatgttaagggcggttttttcctgtttggtcactgatgcctccgtgtaagggggatttctgttcatgggggtaatgataccgatgaaacgagagaggatgctcacgatacgggttactgatgatgaacatgcccggttactggaacgttgtgagggtaaacaactggcggtatggatgcggcgggaccagagaaaaatcactcagggtcaatgccagcgcttcgttaatacagatgtaggtgttccacagggtagccagcagcatcctgcgatgcagatccggaacataatggtgcagggcgctgacttccgcgtttccagactttacgaaacacggaaaccgaagaccattcatgttgttgctcaggtcgcagacgttttgcagcagcagtcgcttcacgttcgctcgcgtatcggtgattcattctgctaaccagtaaggcaaccccgccagcctagccgggtcctcaacgacaggagcacgatcatgcgcacccgtggggccgccatgccggcgataatggcctgcttctcgccgaaacgtttggtggcgggaccagtgacgaaggcttgagcgagggcgtgcaagattccgaataccgcaagcgacaggccgatcatcgtcgcgctccagcgaaagcggtcctcgccgaaaatgacccagagcgctgccggcacctgtcctacgagttgcatgataaagaagacagtcataagtgcggcgacgatagtcatgccccgcgcccaccggaaggagctgactgggttgaaggctctcaagggcatcggtcgagatcccggtgcctaatgagtgagctaacttacattaattgcgttgcgctcactgcccgctttccagtcgggaaacctgtcgtgccagctgcattaatgaatcggccaacgcgcggggagaggcggtttgcgtattgggcgccagggtggtttttcttttcaccagtgagacgggcaacagctgattgcccttcaccgcctggccctgagagagttgcagcaagcggtccacgctggtttgccccagcaggcgaaaatcctgtttgatggtggttaacggcgggatataacatgagctgtcttcggtatcgtcgtatcccactaccgagatatccgcaccaacgcgcagcccggactcggtaatggcgcgcattgcgcccagcgccatctgatcgttggcaaccagcatcgcagtgggaacgatgccctcattcagcatttgcatggtttgttgaaaaccggacatggcactccagtcgccttcccgttccgctatcggctgaatttgattgcgagtgagatatttatgccagccagccagacgcagacgcgccgagacagaacttaatgggcccgctaacagcgcgatttgctggtgacccaatgcgaccagatgctccacgcccagtcgcgtaccgtcttcatgggagaaaataatactgttgatgggtgtctggtcagagacatcaagaaataacgccggaacattagtgcaggcagcttccacagcaatggcatcctggtcatccagcggatagttaatgatcagcccactgacgcgttgcgcgagaagattgtgcaccgccgctttacaggcttcgacgccgcttcgttctaccatcgacaccaccacgctggcacccagttgatcggcgcgagatttaatcgccgcgacaatttgcgacggcgcgtgcagggccagactggaggtggcaacgccaatcagcaacgactgtttgcccgccagttgttgtgccacgcggttgggaatgtaattcagctccgccatcgccgcttccactttttcccgcgttttcgcagaaacgtggctggcctggttcaccacgcgggaaacggtctgataagagacaccggcatactctgcgacatcgtataacgttactggtttcacattcaccaccctgaattgactctcttccgggcgctatcatgccataccgcgaaaggttttgcgccattcgatggtgtccgggatctcgacgctctcccttatgcgactcctgcattaggaagcagcccagtagtaggttgaggccgttgagcaccgccgccgcaaggaatggtgcatgcaaggagatggcgcccaacagtcccccggccacggggcctgccaccatacccacgccgaaacaagcgctcatgagcccgaagtggcgagcccgatcttccccatcggtgatgtcggcgatataggcgccagcaaccgcacctgtggcgccggtgatgccggccacgatgcgtccggcgtagaggatcgagatctcgatcccgcgaaattaatacgactcactataggggaattgtgagcggataacaattcccctctagaaataattttgtttaactttaagaaggagatataccatgggcagcagccatcatcatcatcatcacagcagcggcctggtgccgcgcggcagccatatgatgtcctcacgtaaagagcttgccaatgctattcgtgcgctgagcatggacgcagtacagaaagccaaatccggtcacccgggtgcccctatgggtatggctgacattgccgaagtcctgtggcgtgatttcctgaaacacaacccgcagaatccgtcctgggctgaccgtgaccgcttcgtgctgtccaacggccacggctccatgctgatctacagcctgctgcacctcaccggttacgatctgccgatggaagaactgaaaaacttccgtcagctgcactctaaaactccgggtcacccggaagtgggttacaccgctggtgtggaaaccaccaccggtccgctgggtcagggtattgccaacgcagtcggtatggcgattgcagaaaaaacgctggcggcgcagtttaaccgtccgggccacgacattgtcgaccactacacctacgccttcatgggcgacggctgcatgatggaaggcatctcccacgaagtttgctctctggcgggtacgctgaagctgggtaaactgattgcattctacgatgacaacggtatttctatcgatggtcacgttgaaggctggttcaccgacgacaccgcaatgcgtttcgaagcttacggctggcacgttattcgcgacatcgacggtcatgacgcggcatctatcaaacgcgcagtagaagaagcgcgcgcagtgactgacaaaccttccctgctgatgtgcaaaaccatcatcggtttcggttccccgaacaaagccggtacccacgactcccacggtgcgccgctgggcgacgctgaaattgccctgacccgcgaacaactgggctggaaatatgcgccgttcgaaatcccgtctgaaatctatgctcagtgggatgcgaaagaagcaggccaggcgaaagaatccgcatggaacgagaaattcgctgcttacgcgaaagcttatccgcaggaagccgctgaatttacccgccgtatgaaaggcgaaatgccgtctgacttcgacgctaaagcgaaagagttcatcgctaaactgcaggctaatccggcgaaaatcgccagccgtaaagcgtctcagaatgctatcgaagcgttcggtccgctgttgccggaattcctcggcggttctgctgacctggcgccgtctaacctgaccctgtggtctggttctaaagcaatcaacgaagatgctgcgggtaactacatccactacggtgttcgcgagttcggtatgaccgcgattgctaacggtatctccctgcacggtggcttcctgccgtacacctccaccttcctgatgttcgtggaatacgcacgtaacgccgtacgtatggctgcgctgatgaaacagcgtcaggtgatggtttacacccacgactccatcggtctgggcgaagacggcccgactcaccagccggttgagcaggtcgcttctctgcgcgtaaccccgaacatgtctacatggcgtccgtgtgaccaggttgaatccgcggtcgcgtggaaatacggtgttgagcgtcaggacggcccgaccgcactgatcctctcccgtcagaacctggcgcagcaggaacgaactgaagagcaactggcaaacatcgcgcgcggtggttatgtgctgaaagactgcgccggtcagccggaactgattttcatcgctaccggttcagaagttgaactggctgttgctgcctacgaaaaactgactgccgaaggcgtgaaagcgcgcgtggtgtccatgccgtctaccgacgcatttgacaagcaggatgctgcttaccgtgaatccgtactgccgaaagcggttactgcacgcgttgctgtagaagcgggtattgctgactactggtacaagtatgttggcctgaacggtgctatcgtcggtatgaccaccttcggtgaatctgctccggcagagctgctgtttgaagagttcggcttcactgttgataacgttgttgcgaaagcaaaagaactgctgtaactcgagcaccaccaccaccaccactgagatccggctgctaacaaagcccgaaaggaagctgagttggctgctgccaccgctgagcaataactagcataaccccttggggcctctaaacgggtcttgaggggttttttgctgaaaggaggaactatatccggat

SEQ ID NO: 4 - DNA, 44 bp, Artificial Sequence
  D469T-F
tccatcggtctgggcgaaaccggcccgactcaccagccggttga

SEQ ID NO: 5 - DNA, 44 bp, Artificial Sequence
  D469T-R
ggctggtgagtcgggccggtttcgcccagaccgatggagtcgtg

SEQ ID NO: 6 - DNA, 46 bp, Artificial Sequence
  R520Q-F
accgcactgatcctctcccaacagaacctggcgcagcaggaacgaa

SEQ ID NO: 7 - DNA, 46 bp, Artificial Sequence
  R520Q-R
ctgctgcgccaggttctgttgggagaggatcagtgcggtcgggccg

SEQ ID NO: 8 - DNA, 46 bp, Artificial Sequence
  S385Y-F
tctgctgacctggcgccgtataacctgaccctgtggtctggttcta

SEQ ID NO: 9 - DNA, 46 bp, Artificial Sequence
  S385Y-R
agaccacagggtcaggttatacggcgccaggtcagcagaaccgccg

SEQ ID NO: 10 - DNA, 37 bp, Artificial Sequence
  H26-F
  misc_feature (15)..(15): n is a, c, g or t
  misc_feature (16)..(16): n is a, c, g or t
  misc_feature (17)..(17): k is t or g
aagccaaatccggtnnkccgggtgcccctatgggtat

SEQ ID NO: 11 - DNA, 37 bp, Artificial Sequence
  H26-R
  misc_feature (15)..(15): m is a or c
  misc_feature (16)..(16): n is a, c, g or t
  misc_feature (17)..(17): n is a, c, g or t
ataggggcacccggmnnaccggatttggctttctgta

SEQ ID NO: 12 - DNA, 37 bp, Artificial Sequence
  F434-F
  misc_feature (15)..(15): n is a, c, g or t
  misc_feature (16)..(16): n is a, c, g or t
  misc_feature (17)..(17): k is t or g
cgtacacctccaccnnkctgatgttcgtggaatacgc

SEQ ID NO: 13 - DNA, 37 bp, Artificial Sequence
  F434-R
  misc_feature (15)..(15): m is a or c
  misc_feature (16)..(16): n is a, c, g or t
  misc_feature (17)..(17): n is a, c, g or t
tccacgaacatcagmnnggtggaggtgtacggcagga

SEQ ID NO: 14 - DNA, 37 bp, Artificial Sequence
  L466-F
  misc_feature (15)..(15): n is a, c, g or t
  misc_feature (16)..(16): n is a, c, g or t
  misc_feature (17)..(17): k is t or g
acgactccatcggtnnkggcgaaaccggcccgactca

SEQ ID NO: 15 - DNA, 37 bp, Artificial Sequence
  L466-R
  misc_feature (15)..(15): m is a or c
  misc_feature (16)..(16): n is a, c, g or t
  misc_feature (17)..(17): n is a, c, g or t
gggccggtttcgccmnnaccgatggagtcgtgggtgt

SEQ ID NO: 16 - protein, 663 aa, Artificial Sequence
  Amino acid sequences of E. coli transketolase
MSSRKELANAIRALSMDAVQKAKSGHPGAPMGMADIAEVLWRDFLKHNPQNPSWADRDRFVLSNGHGSMLIYSLLHLTGYDLPMEELKNFRQLHSKTPGHPEVGYTAGVETTTGPLGQGIANAVGMAIAEKTLAAQFNRPGHDIVDHYTYAFMGDGCMMEGISHEVCSLAGTLKLGKLIAFYDDNGISIDGHVEGWFTDDTAMRFEAYGWHVIRDIDGHDAASIKRAVEEARAVTDKPSLLMCKTIIGFGSPNKAGTHDSHGAPLGDAEIALTREQLGWKYAPFEIPSEIYAQWDAKEAGQAKESAWNEKFAAYAKAYPQEAAEFTRRMKGEMPSDFDAKAKEFIAKLQANPAKIASRKASQNAIEAFGPLLPEFLGGSADLAPYNLTLWSGSKAINEDAAGNYIHYGVREFGMTAIANGISLHGGFLPYTSTFLMFVEYARNAVRMAALMKQRQVMVYTHDSIGLGETGPTHQPVEQVASLRVTPNMSTWRPCDQVESAVAWKYGVERQDGPTALILSQQNLAQQERTEEQLANIARGGYVLKDCAGQPELIFIATGSEVELAVAAYEKLTAEGVKARVVSMPSTDAFDKQDAAYRESVLPKAVTARVAVEAGIADYWYKYVGLNGAIVGMTTFGESAPAELLFEEFGFTVDNVVAKAKELL

SEQ ID NO: 17 - DNA, 1992 bp, Artificial Sequence
  Nucleotide sequences of E. coli transketolase
atgtcctcacgtaaagagcttgccaatgctattcgtgcgctgagcatggacgcagtacagaaagccaaatccggtcacccgggtgcccctatgggtatggctgacattgccgaagtcctgtggcgtgatttcctgaaacacaacccgcagaatccgtcctgggctgaccgtgaccgcttcgtgctgtccaacggccacggctccatgctgatctacagcctgctgcacctcaccggttacgatctgccgatggaagaactgaaaaacttccgtcagctgcactctaaaactccgggtcacccggaagtgggttacaccgctggtgtggaaaccaccaccggtccgctgggtcagggtattgccaacgcagtcggtatggcgattgcagaaaaaacgctggcggcgcagtttaaccgtccgggccacgacattgtcgaccactacacctacgccttcatgggcgacggctgcatgatggaaggcatctcccacgaagtttgctctctggcgggtacgctgaagctgggtaaactgattgcattctacgatgacaacggtatttctatcgatggtcacgttgaaggctggttcaccgacgacaccgcaatgcgtttcgaagcttacggctggcacgttattcgcgacatcgacggtcatgacgcggcatctatcaaacgcgcagtagaagaagcgcgcgcagtgactgacaaaccttccctgctgatgtgcaaaaccatcatcggtttcggttccccgaacaaagccggtacccacgactcccacggtgcgccgctgggcgacgctgaaattgccctgacccgcgaacaactgggctggaaatatgcgccgttcgaaatcccgtctgaaatctatgctcagtgggatgcgaaagaagcaggccaggcgaaagaatccgcatggaacgagaaattcgctgcttacgcgaaagcttatccgcaggaagccgctgaatttacccgccgtatgaaaggcgaaatgccgtctgacttcgacgctaaagcgaaagagttcatcgctaaactgcaggctaatccggcgaaaatcgccagccgtaaagcgtctcagaatgctatcgaagcgttcggtccgctgttgccggaattcctcggcggttctgctgacctggcgccgtataacctgaccctgtggtctggttctaaagcaatcaacgaagatgctgcgggtaactacatccactacggtgttcgcgagttcggtatgaccgcgattgctaacggtatctccctgcacggtggcttcctgccgtacacctccaccttcctgatgttcgtggaatacgcacgtaacgccgtacgtatggctgcgctgatgaaacagcgtcaggtgatggtttacacccacgactccatcggtctgggcgaaaccggcccgactcaccagccggttgagcaggtcgcttctctgcgcgtaaccccgaacatgtctacatggcgtccgtgtgaccaggttgaatccgcggtcgcgtggaaatacggtgttgagcgtcaggacggcccgaccgcactgatcctctcccaacagaacctggcgcagcaggaacgaactgaagagcaactggcaaacatcgcgcgcggtggttatgtgctgaaagactgcgccggtcagccggaactgattttcatcgctaccggttcagaagttgaactggctgttgctgcctacgaaaaactgactgccgaaggcgtgaaagcgcgcgtggtgtccatgccgtctaccgacgcatttgacaagcaggatgctgcttaccgtgaatccgtactgccgaaagcggttactgcacgcgttgctgtagaagcgggtattgctgactactggtacaagtatgttggcctgaacggtgctatcgtcggtatgaccaccttcggtgaatctgctccggcagagctgctgtttgaagagttcggcttcactgttgataacgttgttgcgaaagcaaaagaactgctgtaa

SEQ ID NO: 18 - protein, 330 aa, Artificial Sequence
  Amino acid sequences of transaminase ATA117
MAFSADTSEIVYTHDTGLDYITYSDYELDPANPLAGGAAWIEGAFVPPSEARISIFDQGYLHSDVTYTVFHVWNGNAFRLDDHIERLFSNAESMRIIPPLTQDEVKEIALELVAKTELREAFVSVSITRGYSSTPGERDITKHRPQVYMYAVPYQWIVPFDRIRDGVHAMVAQSVRRTPRSSIDPQVKNFQWGDLIRAVQETHDRGFEAPLLLDGDGLLAEGSGFNVVVIKDGVVRSPGRAALPGITRKTVLEIAESLGHEAILADITLAELLDADEVLGCTTAGGVWPFVSVDGNPISDGVPGPVTQSIIRRYWELNVESSSLLTPVQY

SEQ ID NO: 19 - DNA, 990 bp, Artificial Sequence
  Nucleotide sequences of transaminase ATA117
atggcatttagcgcggataccagcgaaatcgtctatacccacgataccggtctggattacatcacctacagcgattacgaactggatccggcaaatccgttagcaggcggcgcagcttggattgaaggcgcatttgttccgccgtctgaagcgcgtattagcatcttcgatcagggctatctgcatagcgacgttacctataccgtcttccacgtttggaacggtaacgcatttcgtctggacgatcacatcgaacgtctgttcagcaacgccgaaagtatgcgtattattccgccgctgacccaagacgaagtcaaagaaatcgcgctggaactggttgcaaaaaccgaactgcgcgaagcgtttgttagcgttagcattacccgcggttatagtagtaccccgggcgaacgcgatattaccaaacatcgtccgcaggtctacatgtacgctgttccgtaccagtggatcgttccgtttgatcgtattcgcgacggcgttcacgcaatggttgcacagagcgtgcgtcgtaccccgcgtagcagcatcgatccgcaggtcaaaaacttccagtggggcgatttaattcgcgcagttcaggaaacccacgatcgcggttttgaagcaccgttactgttagacggcgacggtttactggcagaaggtagcggctttaacgtcgtcgtcattaaagatggggttgttcgttctccgggtcgtgcagcattaccgggtattacccgcaaaaccgttctggaaattgcggaatccctgggtcatgaagcgattctggcggatattaccttagcggaactgctggacgcagacgaagttttaggttgtaccaccgctggcggcgtttggccgtttgttagcgttgacggcaatccgattagcgatggtgttccgggtccggttacccaaagcattattcgtcgctactgggagctgaacgttgaaagtagcagcctgttaaccccggttcagtat